European Patent Application EP 4 714 981 A1, published March 25, 2026. Title: 免疫效应细胞及其应用. Applicant: 科济生物医药（上海）有限公司. The sequence listing filed with the application follows.

SEQUENCE LISTING (55 sequences)

SEQ ID NO: 1 - protein, 21 aa, synthetic construct
  source 1..21: note = signal peptide
MALPVTALLLPLALLLHAARP

SEQ ID NO: 2 - protein, 22 aa, synthetic construct
  source 1..22: note = signal peptide
MLLLVTSLLLCELPHPAFLLIP

SEQ ID NO: 3 - protein, 45 aa, synthetic construct
  source 1..45: note = CD8alpha hinge region
TTTPAPRPPTPAPTIASQPLSLRPEACRPAAGGAVHTRGLDFACD

SEQ ID NO: 4 - protein, 119 aa, synthetic construct
  source 1..119: note = hinge region
ESKYGPPCPPCPGQPREPQVYTLPPSRDELTKNQVSLTCLVKGFYPSDIAVEWESNGQPENNYKTTPPVLDSDGSFFLYSKLTVDKSRWQQGNVFSCSVMHEALHNHYTQKSLSLSPGK

SEQ ID NO: 5 - protein, 228 aa, synthetic construct
  source 1..228: note = hinge region
ESKYGPPCPPCPAPPVAGPSVFLFPPKPKDTLMISRTPEVTCVVVDVSQEDPEVQFNWYVDGVEVHNAKTKPREEQFQSTYRVVSVLTVLHQDWLNGKEYKCKVSNKGLPSSIEKTISKAKGQPREPQVYTLPPSQEEMTKNQVSLTCLVKGFYPSDIAVEWESNGQPENNYKTTPPVLDSDGSFFLYSRLTVDKSRWQEGNVFSCSVMHEALHNHYTQKSLSLSLGK

SEQ ID NO: 6 - protein, 12 aa, synthetic construct
  source 1..12: note = IgG4 short hinge region
ESKYGPPCPPCP

SEQ ID NO: 7 - protein, 24 aa, synthetic construct
  source 1..24: note = CD8 transmembrane region
IYIWAPLAGTCGVLLLSLVITLYC

SEQ ID NO: 8 - protein, 27 aa, synthetic construct
  source 1..27: note = CD28 transmembrane region
FWVLVVVGGVLACYSLLVTVAFIIFWV

SEQ ID NO: 9 - protein, 28 aa, synthetic construct
  source 1..28: note = CD28 transmembrane region
MFWVLVVVGGVLACYSLLVTVAFIIFWV

SEQ ID NO: 10 - protein, 41 aa, synthetic construct
  source 1..41: note = CD28 costimulatory signaling domain
RSKRSRLLHSDYMNMTPRRPGPTRKHYQPYAPPRDFAAYRS

SEQ ID NO: 11 - protein, 42 aa, synthetic construct
  source 1..42: note = CD137 costimulatory signaling domain
KRGRKKLLYIFKQPFMRPVQTTQEEDGCSCRFPEEEEGGCEL

SEQ ID NO: 12 - protein, 113 aa, synthetic construct
  source 1..113: note = CD3zeta signal domain
RVKFSRSADAPAYQQGQNQLYNELNLGRREEYDVLDKRRGRDPEMGGKPQRRKNPQEGLYNELQKDKMAEAYSEIGMKGERRRGKGHDGLYQGLSTATKDTYDALHMQALPPR

SEQ ID NO: 13 - protein, 112 aa, synthetic construct
  source 1..112: note = CD3zeta signal domain
RVKFSRSADAPAYQQGQNQLYNELNLGRREEYDVLDKRRGRDPEMGGKPRRKNPQEGLYNELQKDKMAEAYSEIGMKGERRRGKGHDGLYQGLSTATKDTYDALHMQALPPR

SEQ ID NO: 14 - protein, 15 aa, synthetic construct
  source 1..15: note = linker peptide
GGGGSGGGGSGGGGS

SEQ ID NO: 15 - protein, 18 aa, synthetic construct
  source 1..18: note = linker peptide
GSTSGSGKPGSGEGSTKG

SEQ ID NO: 16 - protein, 5 aa, synthetic construct
  source 1..5: note = linker peptide
GGGGS

SEQ ID NO: 17 - protein, 440 aa, synthetic construct
  source 1..440: note = chimeric receptor sequence
DIQMTQTTSSLSASLGDRVTISCRASQDISKYLNWYQQKPDGTVKLLIYHTSRLHSGVPSRFSGSGSGTDYSLTISNLEQEDIATYFCQQGNTLPYTFGGGTKLEITGSTSGSGKPGSGEGSTKGEVKLQESGPGLVAPSQSLSVTCTVSGVSLPDYGVSWIRQPPRKGLEWLGVIWGSETTYYNSALKSRLTIIKDNSKSQVFLKMNSLQTDDTAIYYCAKHYYYGGSYAMDYWGQGTSVTVSSESKYGPPCPPCPMFWVLVVVGGVLACYSLLVTVAFIIFWVKRGRKKLLYIFKQPFMRPVQTTQEEDGCSCRFPEEEEGGCELRVKFSRSADAPAYQQGQNQLYNELNLGRREEYDVLDKRRGRDPEMGGKPQRRKNPQEGLYNELQKDKMAEAYSEIGMKGERRRGKGHDGLYQGLSTATKDTYDALHMQALPPR

SEQ ID NO: 18 - protein, 19 aa, synthetic construct
  source 1..19: note = P2A linker peptide
ATNFSLLKQAGDVEENPGP

SEQ ID NO: 19 - protein, 22 aa, synthetic construct
  source 1..22: note = F2A linker peptide
VKQTLNFDLLKLAGDVESNPGP

SEQ ID NO: 20 - protein, 20 aa, synthetic construct
  source 1..20: note = E2A linker peptide
QCTNYALLKLAGDVESNPGP

SEQ ID NO: 21 - protein, 120 aa, synthetic construct
  source 1..120: note = CD19 antibody VH
EVKLQESGPGLVAPSQSLSVTCTVSGVSLPDYGVSWIRQPPRKGLEWLGVIWGSETTYYNSALKSRLTIIKDNSKSQVFLKMNSLQTDDTAIYYCAKHYYYGGSYAMDYWGQGTSVTVSS

SEQ ID NO: 22 - protein, 107 aa, synthetic construct
  source 1..107: note = CD19 antibody VL
DIQMTQTTSSLSASLGDRVTISCRASQDISKYLNWYQQKPDGTVKLLIYHTSRLHSGVPSRFSGSGSGTDYSLTISNLEQEDIATYFCQQGNTLPYTFGGGTKLEIT

SEQ ID NO: 23 - protein, 122 aa, synthetic construct
  source 1..122: note = CD20 antibody VH
EVQLVESGGGLVQPGRSLRLSCAASGFTFNDYAMHWVRQAPGKGLEWVSTISWNSGSIGYADSVKGRFTISRDNAKKSLYLQMNSLRAEDTALYYCAKDIQYGNYYYGMDVWGQGTTVTVSS

SEQ ID NO: 24 - protein, 107 aa, synthetic construct
  source 1..107: note = CD20 antibody VL
EIVLTQSPATLSLSPGERATLSCRASQSVSSYLAWYQQKPGQAPRLLIYDASNRATGIPARFSGSGSGTDFTLTISSLEPEDFAVYYCQQRSNWPITFGQGTRLEIK

SEQ ID NO: 25 - protein, 247 aa, synthetic construct
  source 1..247: note = NKG2A antibody scFv
QVQLVQSGAEVKKPGASVKVSCKASGYTFTSYWMNWVRQAPGQGLEWMGRIDPYDSETHYAQKLQGRVTMTTDTSTSTAYMELRSLRSDDTAVYYCARGGYDFDVGTLYWFFDVWGQGTTVTVSSGGGGSGGGGSGGGGSDIQMTQSPSSLSASVGDRVTITCRASENIYSYLAWYQQKPGKAPKLLIYNAKTLAEGVPSRFSGSGSGTDFTLTISSLQPEDFATYYCQHHYGTPRTFGGGTKVEIK

SEQ ID NO: 26 - protein, 243 aa, synthetic construct
  source 1..243: note = FasL antibody scFv
QVQLVQSGAEVKKPGASVKVSCKASGYIFISHGISWVRQAPGQGLEWMGWINAYSGNTNYAQKLQGRVTMTTDRSTSTAYMELRSLRSDDTAVYYCARETMVRGVPCDYWGQGTLVTVSSGGGGSGGGGSGGGGSEIVLTQSPGTLSLSPGERATLSCRASQSVSSSYLAWYQQKPGQAPRLLIYGASSRATGIPDRFSGSGSGTDFTLTISRLEPEDFAVYYCQQYGSSPWTFGQGTKVEIK

SEQ ID NO: 27 - protein, 252 aa, synthetic construct
  source 1..252: note = TIGIT antibody scFv
QVQLVQSGAEVKKPGSSVKVSCKASGGTFSSYAISWVRQAPGQGLEWMGSIIPIFGTANYAQKFQGRVTITADESTSTAYMELSSLRSEDTAVYYCARGPSEVGAILGYVCFDPWGQGTLVTVSSGGGGSGGGGSGGGGSDIVMTQSPLSLPVTPGEPASISCRSSQSLLHSNGYNYLDWYLQKPGQSPQLLIYLGSNRASGVPDRFSGSGSGTDFTLKISRVEAEDVGVYYCMQARRIPITFGGGTKVEIK

SEQ ID NO: 28 - protein, 244 aa, synthetic construct
  source 1..244: note = CD38 antibody scFv
EVQLLESGGGLVQPGGSLRLSCAVSGFTFNSFAMSWVRQAPGKGLEWVSAISGSGGGTYYADSVKGRFTISRDNSKNTLYLQMNSLRAEDTAVYFCAKDKILWFGEPVFDYWGQGTLVTVSSGGGGSGGGGSGGGGSEIVLTQSPATLSLSPGERATLSCRASQSVSSYLAWYQQKPGQAPRLLIYDASNRATGIPARFSGSGSGTDFTLTISSLEPEDFAVYYCQQRSNWPPTFGQGTKVEIK

SEQ ID NO: 29 - protein, 706 aa, synthetic construct
  source 1..706: note = chimeric receptor sequence
DIQMTQTTSSLSASLGDRVTISCRASQDISKYLNWYQQKPDGTVKLLIYHTSRLHSGVPSRFSGSGSGTDYSLTISNLEQEDIATYFCQQGNTLPYTFGGGTKLEIKRGGGGSEVQLVESGGGLVQPGRSLRLSCAASGFTFNDYAMHWVRQAPGKGLEWVSTISWNSGSIGYADSVKGRFTISRDNAKKSLYLQMNSLRAEDTALYYCAKDIQYGNYYYGMDVWGQGTTVTVSSGGGGSGGGGSGGGGSEIVLTQSPATLSLSPGERATLSCRASQSVSSYLAWYQQKPGQAPRLLIYDASNRATGIPARFSGSGSGTDFTLTISSLEPEDFAVYYCQQRSNWPITFGQGTRLEIKGGGGSEVKLQESGPGLVAPSQSLSVTCTVSGVSLPDYGVSWIRQPPRKGLEWLGVIWGSETTYYNSALKSRLTIIKDNSKSQVFLKMNSLQTDDTAIYYCAKHYYYGGSYAMDYWGQGTSVTVSSTTTPAPRPPTPAPTIASQPLSLRPEACRPAAGGAVHTRGLDFACDIYIWAPLAGTCGVLLLSLVITLYCKRGRKKLLYIFKQPFMRPVQTTQEEDGCSCRFPEEEEGGCELRVKFSRSADAPAYQQGQNQLYNELNLGRREEYDVLDKRRGRDPEMGGKPQRRKNPQEGLYNELQKDKMAEAYSEIGMKGERRRGKGHDGLYQGLSTATKDTYDALHMQALPPR

SEQ ID NO: 30 - protein, 706 aa, synthetic construct
  source 1..706: note = chimeric receptor sequence
EIVLTQSPATLSLSPGERATLSCRASQSVSSYLAWYQQKPGQAPRLLIYDASNRATGIPARFSGSGSGTDFTLTISSLEPEDFAVYYCQQRSNWPITFGQGTRLEIKGGGGSEVKLQESGPGLVAPSQSLSVTCTVSGVSLPDYGVSWIRQPPRKGLEWLGVIWGSETTYYNSALKSRLTIIKDNSKSQVFLKMNSLQTDDTAIYYCAKHYYYGGSYAMDYWGQGTSVTVSSGGGGSGGGGSGGGGSDIQMTQTTSSLSASLGDRVTISCRASQDISKYLNWYQQKPDGTVKLLIYHTSRLHSGVPSRFSGSGSGTDYSLTISNLEQEDIATYFCQQGNTLPYTFGGGTKLEIKRGGGGSEVQLVESGGGLVQPGRSLRLSCAASGFTFNDYAMHWVRQAPGKGLEWVSTISWNSGSIGYADSVKGRFTISRDNAKKSLYLQMNSLRAEDTALYYCAKDIQYGNYYYGMDVWGQGTTVTVSSTTTPAPRPPTPAPTIASQPLSLRPEACRPAAGGAVHTRGLDFACDIYIWAPLAGTCGVLLLSLVITLYCKRGRKKLLYIFKQPFMRPVQTTQEEDGCSCRFPEEEEGGCELRVKFSRSADAPAYQQGQNQLYNELNLGRREEYDVLDKRRGRDPEMGGKPQRRKNPQEGLYNELQKDKMAEAYSEIGMKGERRRGKGHDGLYQGLSTATKDTYDALHMQALPPR

SEQ ID NO: 31 - protein, 709 aa, synthetic construct
  source 1..709: note = chimeric receptor sequence
DIQMTQTTSSLSASLGDRVTISCRASQDISKYLNWYQQKPDGTVKLLIYHTSRLHSGVPSRFSGSGSGTDYSLTISNLEQEDIATYFCQQGNTLPYTFGGGTKLEIKRGGGGSEVQLVESGGGLVQPGRSLRLSCAASGFTFNDYAMHWVRQAPGKGLEWVSTISWNSGSIGYADSVKGRFTISRDNAKKSLYLQMNSLRAEDTALYYCAKDIQYGNYYYGMDVWGQGTTVTVSSGSTSGSGKPGSGEGSTKGEIVLTQSPATLSLSPGERATLSCRASQSVSSYLAWYQQKPGQAPRLLIYDASNRATGIPARFSGSGSGTDFTLTISSLEPEDFAVYYCQQRSNWPITFGQGTRLEIKGGGGSEVKLQESGPGLVAPSQSLSVTCTVSGVSLPDYGVSWIRQPPRKGLEWLGVIWGSETTYYNSALKSRLTIIKDNSKSQVFLKMNSLQTDDTAIYYCAKHYYYGGSYAMDYWGQGTSVTVSSTTTPAPRPPTPAPTIASQPLSLRPEACRPAAGGAVHTRGLDFACDIYIWAPLAGTCGVLLLSLVITLYCKRGRKKLLYIFKQPFMRPVQTTQEEDGCSCRFPEEEEGGCELRVKFSRSADAPAYQQGQNQLYNELNLGRREEYDVLDKRRGRDPEMGGKPQRRKNPQEGLYNELQKDKMAEAYSEIGMKGERRRGKGHDGLYQGLSTATKDTYDALHMQALPPR

SEQ ID NO: 32 - protein, 679 aa, synthetic construct
  source 1..679: note = chimeric receptor sequence
DIQMTQTTSSLSASLGDRVTISCRASQDISKYLNWYQQKPDGTVKLLIYHTSRLHSGVPSRFSGSGSGTDYSLTISNLEQEDIATYFCQQGNTLPYTFGGGTKLEITGGGGSEVQLVESGGGLVQPGRSLRLSCAASGFTFNDYAMHWVRQAPGKGLEWVSTISWNSGSIGYADSVKGRFTISRDNAKKSLYLQMNSLRAEDTALYYCAKDIQYGNYYYGMDVWGQGTTVTVSSGSTSGSGKPGSGEGSTKGEIVLTQSPATLSLSPGERATLSCRASQSVSSYLAWYQQKPGQAPRLLIYDASNRATGIPARFSGSGSGTDFTLTISSLEPEDFAVYYCQQRSNWPITFGQGTRLEIKGGGGSEVKLQESGPGLVAPSQSLSVTCTVSGVSLPDYGVSWIRQPPRKGLEWLGVIWGSETTYYNSALKSRLTIIKDNSKSQVFLKMNSLQTDDTAIYYCAKHYYYGGSYAMDYWGQGTSVTVSSESKYGPPCPPCPMFWVLVVVGGVLACYSLLVTVAFIIFWVKRGRKKLLYIFKQPFMRPVQTTQEEDGCSCRFPEEEEGGCELRVKFSRSADAPAYQQGQNQLYNELNLGRREEYDVLDKRRGRDPEMGGKPQRRKNPQEGLYNELQKDKMAEAYSEIGMKGERRRGKGHDGLYQGLSTATKDTYDALHMQALPPR

SEQ ID NO: 33 - protein, 679 aa, synthetic construct
  source 1..679: note = chimeric receptor sequence
EVKLQESGPGLVAPSQSLSVTCTVSGVSLPDYGVSWIRQPPRKGLEWLGVIWGSETTYYNSALKSRLTIIKDNSKSQVFLKMNSLQTDDTAIYYCAKHYYYGGSYAMDYWGQGTSVTVSSGGGGSEIVLTQSPATLSLSPGERATLSCRASQSVSSYLAWYQQKPGQAPRLLIYDASNRATGIPARFSGSGSGTDFTLTISSLEPEDFAVYYCQQRSNWPITFGQGTRLEIKGSTSGSGKPGSGEGSTKGEVQLVESGGGLVQPGRSLRLSCAASGFTFNDYAMHWVRQAPGKGLEWVSTISWNSGSIGYADSVKGRFTISRDNAKKSLYLQMNSLRAEDTALYYCAKDIQYGNYYYGMDVWGQGTTVTVSSGGGGSDIQMTQTTSSLSASLGDRVTISCRASQDISKYLNWYQQKPDGTVKLLIYHTSRLHSGVPSRFSGSGSGTDYSLTISNLEQEDIATYFCQQGNTLPYTFGGGTKLEITESKYGPPCPPCPMFWVLVVVGGVLACYSLLVTVAFIIFWVKRGRKKLLYIFKQPFMRPVQTTQEEDGCSCRFPEEEEGGCELRVKFSRSADAPAYQQGQNQLYNELNLGRREEYDVLDKRRGRDPEMGGKPQRRKNPQEGLYNELQKDKMAEAYSEIGMKGERRRGKGHDGLYQGLSTATKDTYDALHMQALPPR

SEQ ID NO: 34 - protein, 716 aa, synthetic construct
  source 1..716: note = chimeric receptor sequence
EVQLVESGGGLVQPGRSLRLSCAASGFTFNDYAMHWVRQAPGKGLEWVSTISWNSGSIGYADSVKGRFTISRDNAKKSLYLQMNSLRAEDTALYYCAKDIQYGNYYYGMDVWGQGTTVTVSSGGGGSGGGGSGGGGSEIVLTQSPATLSLSPGERATLSCRASQSVSSYLAWYQQKPGQAPRLLIYDASNRATGIPARFSGSGSGTDFTLTISSLEPEDFAVYYCQQRSNWPITFGQGTRLEIKGGGGSDIQMTQTTSSLSASLGDRVTISCRASQDISKYLNWYQQKPDGTVKLLIYHTSRLHSGVPSRFSGSGSGTDYSLTISNLEQEDIATYFCQQGNTLPYTFGGGTKLEIKRGGGGSGGGGSGGGGSEVKLQESGPGLVAPSQSLSVTCTVSGVSLPDYGVSWIRQPPRKGLEWLGVIWGSETTYYNSALKSRLTIIKDNSKSQVFLKMNSLQTDDTAIYYCAKHYYYGGSYAMDYWGQGTSVTVSSTTTPAPRPPTPAPTIASQPLSLRPEACRPAAGGAVHTRGLDFACDIYIWAPLAGTCGVLLLSLVITLYCKRGRKKLLYIFKQPFMRPVQTTQEEDGCSCRFPEEEEGGCELRVKFSRSADAPAYQQGQNQLYNELNLGRREEYDVLDKRRGRDPEMGGKPQRRKNPQEGLYNELQKDKMAEAYSEIGMKGERRRGKGHDGLYQGLSTATKDTYDALHMQALPPR

SEQ ID NO: 35 - DNA, 20 bp, synthetic construct
  source 1..20: mol_type = other DNA; note = coding sequence of sgRNA
agagtctctcagctggtaca

SEQ ID NO: 36 - DNA, 20 bp, synthetic construct
  source 1..20: mol_type = other DNA; note = coding sequence of sgRNA
gagtagcgcgagcacagcta

SEQ ID NO: 37 - DNA, 20 bp, synthetic construct
  source 1..20: mol_type = other DNA; note = coding sequence of sgRNA
gcacttggtattctgggtcc

SEQ ID NO: 38 - DNA, 20 bp, synthetic construct
  source 1..20: mol_type = other DNA; note = coding sequence of sgRNA
tgaacaggaaataacctatg

SEQ ID NO: 39 - protein, 224 aa, synthetic construct
  source 1..224: note = chimeric receptor sequence
TTTPAPRPPTPAPTIASQPLSLRPEACRPAAGGAVHTRGLDFACDIYIWAPLAGTCGVLLLSLVITLYCKRGRKKLLYIFKQPFMRPVQTTQEEDGCSCRFPEEEEGGCELRVKFSRSADAPAYQQGQNQLYNELNLGRREEYDVLDKRRGRDPEMGGKPQRRKNPQEGLYNELQKDKMAEAYSEIGMKGERRRGKGHDGLYQGLSTATKDTYDALHMQALPPR

SEQ ID NO: 40 - protein, 195 aa, synthetic construct
  source 1..195: note = chimeric receptor sequence
ESKYGPPCPPCPMFWVLVVVGGVLACYSLLVTVAFIIFWVKRGRKKLLYIFKQPFMRPVQTTQEEDGCSCRFPEEEEGGCELRVKFSRSADAPAYQQGQNQLYNELNLGRREEYDVLDKRRGRDPEMGGKPQRRKNPQEGLYNELQKDKMAEAYSEIGMKGERRRGKGHDGLYQGLSTATKDTYDALHMQALPPR

SEQ ID NO: 41 - protein, 194 aa, synthetic construct
  source 1..194: note = chimeric receptor sequence
ESKYGPPCPPCPMFWVLVVVGGVLACYSLLVTVAFIIFWVRSKRSRLLHSDYMNMTPRRPGPTRKHYQPYAPPRDFAAYRSRVKFSRSADAPAYQQGQNQLYNELNLGRREEYDVLDKRRGRDPEMGGKPQRRKNPQEGLYNELQKDKMAEAYSEIGMKGERRRGKGHDGLYQGLSTATKDTYDALHMQALPPR

SEQ ID NO: 42 - protein, 226 aa, synthetic construct
  source 1..226: note = chimeric receptor sequence
TTTPAPRPPTPAPTIASQPLSLRPEACRPAAGGAVHTRGLDFACDFWVLVVVGGVLACYSLLVTVAFIIFWVRSKRSRLLHSDYMNMTPRRPGPTRKHYQPYAPPRDFAAYRSRVKFSRSADAPAYQQGQNQLYNELNLGRREEYDVLDKRRGRDPEMGGKPQRRKNPQEGLYNELQKDKMAEAYSEIGMKGERRRGKGHDGLYQGLSTATKDTYDALHMQALPPR

SEQ ID NO: 43 - protein, 5 aa, synthetic construct
  source 1..5: note = VH-CDR1
DYGVS

SEQ ID NO: 44 - protein, 16 aa, synthetic construct
  source 1..16: note = VH-CDR2
VIWGSETTYYNSALKS

SEQ ID NO: 45 - protein, 12 aa, synthetic construct
  source 1..12: note = VH-CDR3
HYYYGGSYAMDY

SEQ ID NO: 46 - protein, 11 aa, synthetic construct
  source 1..11: note = VL-CDR1
RASQDISKYLN

SEQ ID NO: 47 - protein, 7 aa, synthetic construct
  source 1..7: note = VL-CDR2
HTSRLHS

SEQ ID NO: 48 - protein, 9 aa, synthetic construct
  source 1..9: note = VL-CDR3
QQGNTLPYT

SEQ ID NO: 49 - protein, 5 aa, synthetic construct
  source 1..5: note = VH-CDR1
DYAMH

SEQ ID NO: 50 - protein, 17 aa, synthetic construct
  source 1..17: note = VH-CDR2
TISWNSGSIGYADSVKG

SEQ ID NO: 51 - protein, 13 aa, synthetic construct
  source 1..13: note = VH-CDR3
DIQYGNYYYGMDV

SEQ ID NO: 52 - protein, 11 aa, synthetic construct
  source 1..11: note = VL-CDR1
RASQSVSSYLA

SEQ ID NO: 53 - protein, 7 aa, synthetic construct
  source 1..7: note = VL-CDR2
DASNRAT

SEQ ID NO: 54 - protein, 9 aa, synthetic construct
  source 1..9: note = VL-CDR3
QQRSNWPIT

SEQ ID NO: 55 - protein, 442 aa, synthetic construct
  source 1..442: note = chimeric receptor sequence
EVQLVESGGGLVQPGRSLRLSCAASGFTFNDYAMHWVRQAPGKGLEWVSTISWNSGSIGYADSVKGRFTISRDNAKKSLYLQMNSLRAEDTALYYCAKDIQYGNYYYGMDVWGQGTTVTVSSGSTSGGGSGGGSGGGGSSEIVLTQSPATLSLSPGERATLSCRASQSVSSYLAWYQQKPGQAPRLLIYDASNRATGIPARFSGSGSGTDFTLTISSLEPEDFAVYYCQQRSNWPITFGQGTRLEIKESKYGPPCPPCPMFWVLVVVGGVLACYSLLVTVAFIIFWVKRGRKKLLYIFKQPFMRPVQTTQEEDGCSCRFPEEEEGGCELRVKFSRSADAPAYQQGQNQLYNELNLGRREEYDVLDKRRGRDPEMGGKPQRRKNPQEGLYNELQKDKMAEAYSEIGMKGERRRGKGHDGLYQGLSTATKDTYDALHMQALPPR